European Patent Specification EP 3 898 668 B1, published August 30, 2023. Title: ANTIBODIES THAT NEUTRALIZE HEPATITIS B VIRUS AND USES THEREOF. Applicant: Humabs BioMed SA Corti, Davide. Application PCT. The sequence listing filed with the application follows.

SEQUENCE LISTING (139 sequences)

SEQ ID NO: 1 - protein, 11 aa, Hepatitus B virus
  VARIANT (1)...(11): Xaa = any amino acid
XXXTCXXXAXG

SEQ ID NO: 2 - protein, 11 aa, Hepatitus B Virus
  VARIANT 1: Xaa = P, T or S,
  VARIANT 2: Xaa = C or S,
  VARIANT 3: Xaa = R, K, D or I,
  VARIANT 6: Xaa = M or T
  VARIANT 7: Xaa = T, A or I
  VARIANT 8: Xaa = T, P or L
  VARIANT (10)...(10): Xaa = Q, H or L.
XXXTCXXXAXG

SEQ ID NO: 3 - protein, 226 aa, Hepatitis B Virus
  S domain of HBsAg (GenBank acc. no. J02203)
MENITSGFLGPLLVLQAGFFLLTRILTIPQSLDSWWTSLNFLGGTTVCLGQNSQSPTSNHSPTSCPPTCPGYRWMCLRRFIIFLFILLLCLIFLLVLLDYQGMLPVCPLIPGSSTTSTGPCRTCMTTAQGTSMYPSCCCTKPSDGNCTCIPIPSSWAFGKFLWEWASARFSWLSLLVPFVQWFVGLSPTVWLSVIWMMWYWGPSLYSILSPFLPLLPIFFCLWVYI

SEQ ID NO: 4 - protein, 226 aa, Hepatits B Virus
  S domain of HBsAg (GenBank acc. no. FJ899792)
MENVTSGFLGPLLVLQAGFFLLTRILTIPQSLDSWWTSLNFLGGTTVCLGQNSQSPTSNHSPTSCPPTCPGYRWMCLRRFIIFLFILLLCLIFLLVLLDYQGMLPVCPLIPGSSTTGTGPCRTCTTPAQGTSMYPSCCCTKPSDGNCTCIPIPSSWAFGKFLWEWASARFSWLSLLVPFVQWFVGLSPTVWLSVIWMMWYWGPSLYSTLSPFLPLLPIFFCLWVYI

SEQ ID NO: 5 - protein, 72 aa, Hepatitis B Virus
  J02203 (D, ayw3)
QGMLPVCPLIPGSSTTSTGPCRTCMTTAQGTSMYPSCCCTKPSDGNCTCIPIPSSWAFGKFLWEWASARFSW

SEQ ID NO: 6 - protein, 72 aa, Hepatitis B Virus
  FJ899792 (D, adw2)
QGMLPVCPLIPGSSTTGTGPCRTCTTPAQGTSMYPSCCCTKPSDGNCTCIPIPSSWAFGKFLWEWASARFSW

SEQ ID NO: 7 - protein, 72 aa, Hepatitis B Virus
  AM282986 (A)
QGMLPVCPLIPGTTTTSTGPCKTCTTPAQGNSMFPSCCCTKPSDGNCTCIPIPSSWAFAKYLWEWASVRFSW

SEQ ID NO: 8 - protein, 72 aa, Hepatitis B Virus
  D23678 (B1)
QGMLPVCPLIPGSSTTSTGPCKTCTTPAQGTSMFPSCCCTKPTDGNCTCIPIPSSWAFAKYLWEWASVRFSW

SEQ ID NO: 9 - protein, 72 aa, Hepatitis B Virus
  AB117758 (C1)
QGMLPVCPLLPGTSTTSTGPCKTCTIPAQGTSMFPSCCCTKPSDGNCTCIPIPSSWAFARFLWEWASVRFSW

SEQ ID NO: 10 - protein, 72 aa, Hepatitis B Virus
  AB205192 (E)
QGMLPVCPLIPGSSTTSTGPCRTCTTLAQGTSMFPSCCCSKPSDGNCTCIPIPSSWAFGKFLWEWASARFSW

SEQ ID NO: 11 - protein, 72 aa, Hepatitis B Virus
  X69798 (F4)
QGMLPVCPLLPGSTTTSTGPCKTCTTLAQGTSMFPSCCCSKPSDGNCTCIPIPSSWALGKYLWEWASARFSW

SEQ ID NO: 12 - protein, 72 aa, Hepatitis B Virus
  AF160501 (G)
QGMLPVCPLIPGSSTTSTGPCKTCTTPAQGNSMYPSCCCTKPSDGNCTCIPIPSSWAFAKYLWEWASVRFSW

SEQ ID NO: 13 - protein, 72 aa, Hepatitis B Virus
  AY090454 (H)
QGMLPVCPLLPGSTTTSTGPCKTCTTLAQGTSMFPSCCCTKPSDGNCTCIPIPSSWAFGKYLWEWASARFSW

SEQ ID NO: 14 - protein, 72 aa, Hepatitis B Virus
  AF241409 (I)
QGMLPVCPLIPGSSTTSTGPCKTCTTPAQGNSMYPSCCCTKPSDGNCTCIPIPSSWAFAKYLWEWASARFSW

SEQ ID NO: 15 - protein, 72 aa, Hepatitis B Virus
  AB486012 (J)
QGMLPVCPLLPGSTTTSTGPCRTCTITAQGTSMFPSCCCTKPSDGNCTCIPIPSSWAFAKFLWEWASVRFSW

SEQ ID NO: 16 - protein, 73 aa, Hepatitis B Virus
  HBsAg Y100C/P120T
CQGMLPVCPLIPGSSTTGTGTCRTCTTPAQGTSMYPSCCCTKPSDGNCTCIPIPSSWAFGKFLWEWASARFSW

SEQ ID NO: 17 - protein, 72 aa, Hepatitis B Virus
  HBsAg P120T
QGMLPVCPLIPGSSTTGTGTCRTCTTPAQGTSMYPSCCCTKPSDGNCTCIPIPSSWAFGKFLWEWASARFSW

SEQ ID NO: 18 - protein, 72 aa, Hepatitis B Virus
  HBsAg P120T/S143L
QGMLPVCPLIPGSSTTGTGTCRTCTTPAQGTSMYPSCCCTKPLDGNCTCIPIPSSWAFGKFLWEWASARFSW

SEQ ID NO: 19 - protein, 72 aa, Hepatitis B Virus
  HBsAg C121S
QGMLPVCPLIPGSSTTGTGPSRTCTTPAQGTSMYPSCCCTKPSDGNCTCIPIPSSWAFGKFLWEWASARFSW

SEQ ID NO: 20 - protein, 72 aa, Hepatitis B Virus
  HBsAg R122D
QGMLPVCPLIPGSSTTGTGPCDTCTTPAQGTSMYPSCCCTKPSDGNCTCIPIPSSWAFGKFLWEWASARFSW

SEQ ID NO: 21 - protein, 72 aa, Hepatitis B Virus
  HBsAg R122I
QGMLPVCPLIPGSSTTGTGPCITCTTPAQGTSMYPSCCCTKPSDGNCTCIPIPSSWAFGKFLWEWASARFSW

SEQ ID NO: 22 - protein, 72 aa, Hepatitis B Virus
  HBsAg T123N
QGMLPVCPLIPGSSTTGTGPCRNCTTPAQGTSMYPSCCCTKPSDGNCTCIPIPSSWAFGKFLWEWASARFSW

SEQ ID NO: 23 - protein, 72 aa, Hepatitis B Virus
  HBsAg Q129H
QGMLPVCPLIPGSSTTGTGPCRTCTTPAHGTSMYPSCCCTKPSDGNCTCIPIPSSWAFGKFLWEWASARFSW

SEQ ID NO: 24 - protein, 72 aa, Hepatitis B Virus
  HBsAg Q129L
QGMLPVCPLIPGSSTTGTGPCRTCTTPALGTSMYPSCCCTKPSDGNCTCIPIPSSWAFGKFLWEWASARFSW

SEQ ID NO: 25 - protein, 72 aa, Hepatitis B Virus
  HBsAg M133H
QGMLPVCPLIPGSSTTGTGPCRTCTTPAQGTSHYPSCCCTKPSDGNCTCIPIPSSWAFGKFLWEWASARFSW

SEQ ID NO: 26 - protein, 72 aa, Hepatitis B Virus
  HBsAg M133L
QGMLPVCPLIPGSSTTGTGPCRTCTTPAQGTSLYPSCCCTKPSDGNCTCIPIPSSWAFGKFLWEWASARFSW

SEQ ID NO: 27 - protein, 72 aa, Hepatitis B Virus
  HBsAg M133T
QGMLPVCPLIPGSSTTGTGPCRTCTTPAQGTSTYPSCCCTKPSDGNCTCIPIPSSWAFGKFLWEWASARFSW

SEQ ID NO: 28 - protein, 72 aa, Hepatitis B Virus
  HBsAg K141E
QGMLPVCPLIPGSSTTGTGPCRTCTTPAQGTSMYPSCCCTEPSDGNCTCIPIPSSWAFGKFLWEWASARFSW

SEQ ID NO: 29 - protein, 72 aa, Hepatitis B Virus
  HBsAg P142S
QGMLPVCPLIPGSSTTGTGPCRTCTTPAQGTSMYPSCCCTKSSDGNCTCIPIPSSWAFGKFLWEWASARFSW

SEQ ID NO: 30 - protein, 72 aa, Hepatitis B Virus
  HBsAg S143K
QGMLPVCPLIPGSSTTGTGPCRTCTTPAQGTSMYPSCCCTKPKDGNCTCIPIPSSWAFGKFLWEWASARFSW

SEQ ID NO: 31 - protein, 72 aa, Hepatitis B Virus
  HBsAg D144A
QGMLPVCPLIPGSSTTGTGPCRTCTTPAQGTSMYPSCCCTKPSAGNCTCIPIPSSWAFGKFLWEWASARFSW

SEQ ID NO: 32 - protein, 72 aa, Hepatitis B Virus
  HBsAg G145R
QGMLPVCPLIPGSSTTGTGPCRTCTTPAQGTSMYPSCCCTKPSDRNCTCIPIPSSWAFGKFLWEWASARFSW

SEQ ID NO: 33 - protein, 72 aa, Hepatitis B Virus
  HBsAg N146A
QGMLPVCPLIPGSSTTGTGPCRTCTTPAQGTSMYPSCCCTKPSDGACTCIPIPSSWAFGKFLWEWASARFSW

SEQ ID NO: 34 - protein, 8 aa, Artificial Sequence
  Synthetic sequence HBC34 CDRH1
GRIFRSFY

SEQ ID NO: 35 - protein, 7 aa, Artificial Sequence
  Synthetic sequence HBC34 CDRH2
NQDGSEK

SEQ ID NO: 36 - protein, 12 aa, Artificial Sequence
  Synthetic sequence HBC34 CDRH3
AAWSGNSGGMDV

SEQ ID NO: 37 - protein, 6 aa, Artificial Sequence
  Synthetic sequence HBC34 CDRL1
KLGNKN

SEQ ID NO: 38 - protein, 3 aa, Artificial Sequence
  Synthetic sequence HBC34 CDRL2
EVK

SEQ ID NO: 39 - protein, 9 aa, Artificial Sequence
  Synthetic sequence HBC34 CDRL2 long
VIYEVKYRP

SEQ ID NO: 40 - protein, 9 aa, Artificial Sequence
  Synthetic sequence HBC34 CDRL3
QTWDSTTVV

SEQ ID NO: 41 - protein, 119 aa, Artificial Sequence
  Synthetic sequence HBC34, HBC34-V7, HBC34-V34, HBC34-V35 VH
ELQLVESGGGWVQPGGSQRLSCAASGRIFRSFYMSWVRQAPGKGLEWVATINQDGSEKLYVDSVKGRFTISRDNAKNSLFLQMNNLRVEDTAVYYCAAWSGNSGGMDVWGQGTTVSVSS

SEQ ID NO: 42 - protein, 106 aa, Artificial Sequence
  Synthetic sequence HBC34 VL
SYELTQPPSVSVSPGQTVSIPCSGDKLGNKNVCWFQHKPGQSPVLVIYEVKYRPSGIPERFSGSNSGNTATLTISGTQAMDEAAYFCQTWDSTTVVFGGGTRLTVL

SEQ ID NO: 43 - DNA, 24 bp, Artificial Sequence
  Synthetic sequence HBC34 CDRH1
ggacgcatctttagaagtttttac

SEQ ID NO: 44 - DNA, 24 bp, Artificial Sequence
  Synthetic sequence HBC34 CDRH2
ataaaccaagatggaagtgagaaa

SEQ ID NO: 45 - DNA, 36 bp, Artificial Sequence
  Synthetic sequence HBC34 CDRH3
gcggcttggagcggcaatagtgggggtatggacgtc

SEQ ID NO: 46 - DNA, 18 bp, Artificial Sequence
  Synthetic sequence HBC34 CDRL1
aaattggggaataaaaat

SEQ ID NO: 47 - DNA, 9 bp, Artificial Sequence
  Synthetic sequence HBC34 CDRL2
gaggttaaa

SEQ ID NO: 48 - DNA, 27 bp, Artificial Sequence
  Synthetic sequence HBC34 CDRL2 long
gtcatctatgaggttaaataccgcccc

SEQ ID NO: 49 - DNA, 27 bp, Artificial Sequence
  Synthetic sequence HBC34 CDRL3
cagacgtgggacagcaccactgtggtg

SEQ ID NO: 50 - DNA, 357 bp, Artificial Sequence
  Synthetic sequence HBC34 VH
gaactgcagctggtggagtctgggggaggctgggtccagccgggggggtcccagagactgtcctgtgcagcctctggacgcatctttagaagtttttacatgagctgggtccgccaggccccagggaaggggctggagtgggtggccactataaaccaagatggaagtgagaaattatatgtggactctgtgaagggccgattcaccatctccagagacaacgccaagaactcactatttctgcaaatgaacaacctgagagtcgaggacacggccgtttattactgcgcggcttggagcggcaatagtgggggtatggacgtctggggccaggggaccacggtctccgtctcctca

SEQ ID NO: 51 - DNA, 318 bp, Artificial Sequence
  Synthetic sequence HBC34 VL
tcctatgagctgactcagccaccctcagtgtccgtgtccccaggacagacagtcagcatcccctgctctggagataaattggggaataaaaatgtttgctggtttcagcataagccaggccagtcccctgtgttggtcatctatgaggttaaataccgcccctcggggattcctgagcgattctctggctccaactctgggaacacagccactctgaccatcagcgggacccaggctatggatgaggctgcctatttctgtcagacgtgggacagcaccactgtggtgttcggcggagggaccaggctgaccgtccta

SEQ ID NO: 52 - protein, 33 aa, Hepatitis B Virus
  VARIANT (1)...(33): Xaa = Any Amino Acid
XGSSTTSTGPCRTCMTXPSDGNATAIPIPSSWX

SEQ ID NO: 53 - protein, 15 aa, Hepatitis B Virus
TSTGPCRTCMTTAQG

SEQ ID NO: 54 - protein, 26 aa, Hepatitis B Virus
GMLPVCPLIPGSSTTSTGPCRTCMTT

SEQ ID NO: 55 - protein, 33 aa, Hepatitis B Virus
  VARIANT (1)...(33): Xaa = Any Amino Acid
XSMYPSASATKPSDGNXTGPCRTCMTTAQGTSX

SEQ ID NO: 56 - protein, 11 aa, Hepatitis B Virus
  amino acids 120 - 130 of the S domain of HBsAg (HBV-D J02203)
PCRTCMTTAQG

SEQ ID NO: 57 - protein, 11 aa, Hepatitis B Virus
  VARIANT 3: Xaa = R or K
  VARIANT 6: Xaa = M or T
  VARIANT 7: Xaa = T or I
  VARIANT 8: Xaa = T, P or L
PCXTCXXXAQG

SEQ ID NO: 58 - protein, 9 aa, Artificial Sequence
  Synthetic sequence HBC34-V7 CDRL3 and HBC34-V23 CDRL3
QTFDSTTVV

SEQ ID NO: 59 - protein, 106 aa, Artificial Sequence
  Synthetic sequence HBC34-V7 VL
SYELTQPPSVSVSPGQTVSIPCSGDKLGNKNVCWFQHKPGQSPVLVIYEVKYRPSGIPERFSGSNSGNTATLTISGTQAMDEAAYFCQTFDSTTVVFGGGTRLTVL

SEQ ID NO: 60 - DNA, 18 bp, Artificial Sequence
  Synthetic sequence HBC34v7 CDRL1 and HBC-V23 CDRL1
aagctggggaacaaaaat

SEQ ID NO: 61 - DNA, 9 bp, Artificial Sequence
  Synthetic sequence HBC34-V7 CDRL2 and HBC34v23 CDRL2
gaggtgaaa

SEQ ID NO: 62 - DNA, 27 bp, Artificial Sequence
  Synthetic sequence HBC34-V7 CDRL2 long and CDRL2 HBC34-V23 long
gtcatctacgaggtgaaatatcggcct

SEQ ID NO: 63 - DNA, 27 bp, Artificial Sequence
  Synthetic sequence CDRL3 HBC34-V7 and CDRL3 HBC34-V23
cagacattcgattccaccacagtggtc

SEQ ID NO: 64 - DNA, 318 bp, Artificial Sequence
  Synthetic sequence HBC34-V7, HBC34-V34, and HBC34-V35 VL
tcttacgagctgacacagccacctagcgtgtccgtctctccaggacagaccgtgtccatcccttgctctggcgacaagctggggaacaaaaatgtctgttggttccagcacaagccagggcagagtcccgtgctggtcatctacgaggtgaaatatcggccttcaggaattccagaacggttcagcggatcaaacagcggcaatactgcaaccctgacaattagcgggacccaggccatggacgaagccgcttatttctgccagacattcgattccaccacagtggtctttggcgggggaactaggctgaccgtgctg

SEQ ID NO: 65 - protein, 106 aa, Artificial Sequence
  Synthetic sequence HBC34-V23 VL
SYELTQPPSVSVSPGQTASITCSGDKLGNKNACWYQQKPGQSPVLVIYEVKYRPSGIPERFSGSNSGNTATLTISGTQAMDEADYYCQTFDSTTVVFGGGTKLTVL

SEQ ID NO: 66 - protein, 8 aa, Artificial Sequence
  Synthetic sequence HBC34wt CDRH2
INQDGSEK

SEQ ID NO: 67 - protein, 119 aa, Artificial Sequence
  Synthetic sequence HBC34-V31, HBC34-V32 and HBC34-V33 VH
EVQLVESGGGLVQPGGSLRLSCAASGRIFRSFYMSWVRQAPGKGLEWVANINQDGSEKLYVDSVKGRFTISRDNAKNSLFLQMNNLRVEDTAVYYCAAWSGNSGGMDVWGQGTTVTVSS

SEQ ID NO: 68 - DNA, 357 bp, Artificial Sequence
  Synthetic sequence HBC34-V31, HBC34-V32 and HBC34-V33 VH
gaggtgcagctggtggaatccggcgggggactggtgcagcctggcggctcactgagactgagctgtgcagcttctggaagaatcttcagatctttttacatgagttgggtgagacaggctcctgggaagggactggagtgggtcgcaaacatcaatcaggacggatcagaaaagctgtatgtggatagcgtcaaaggcaggttcactatttcccgcgacaacgccaaaaattctctgtttctgcagatgaacaatctgcgggtggaggataccgctgtctactattgtgcagcctggtctggcaacagtggaggcatggacgtgtggggacagggaaccacagtgacagtcagctcc

SEQ ID NO: 69 - DNA, 318 bp, Artificial Sequence
  Synthetic sequence HBC34v23 VL
tcttacgagctgacacagccccctagcgtgtccgtctctccaggccagacagcatccatcacttgctctggcgacaagctggggaacaaaaatgcctgttggtatcagcagaagccagggcagagtcccgtgctggtcatctacgaggtgaaatatcggccttcaggaattccagaaagattcagtggatcaaacagcggcaatactgctaccctgacaattagcgggacccaggccatggacgaagctgattactattgccagacattcgattccaccacagtggtctttggcgggggaactaagctgaccgtgctg

SEQ ID NO: 70 - DNA, 357 bp, Artificial Sequence
  Synthetic sequence HBC34 wt VH codon optimized
gaactgcagctggtcgaatcaggaggagggtgggtccagcccggagggagccagagactgtcttgtgccgcatcagggaggatcttcaggagcttctacatgtcctgggtgcgccaggcaccaggcaagggactggagtgggtcgccaccatcaaccaggacggatctgaaaagctgtatgtggatagtgtcaaaggccggttcacaattagcagagacaacgctaaaaattctctgtttctgcagatgaacaatctgcgagtggaggataccgccgtctactattgcgccgcttggtctggcaacagcggcgggatggatgtctgggggcagggcacaacagtgagcgtctcttcc

SEQ ID NO: 71 - DNA, 318 bp, Artificial Sequence
  Synthetic sequence HBC34 wt VL codon optimized
tcatacgaactgactcagcctccctccgtctccgtctcacctggacagaccgtctcaatcccctgctccggcgataaactgggcaacaagaacgtgtgctggttccagcacaaacccggacagagtcctgtgctggtcatctacgaggtcaagtatcggccaagcggcattcccgaaagattcagcggctccaactctgggaataccgcaacactgactatctctggaacccaggcaatggacgaggcagcttacttttgccagacttgggattcaactactgtcgtgttcggcggcggaactagactgactgtcctg

SEQ ID NO: 72 - DNA, 24 bp, Artificial Sequence
  Synthetic sequence HBC34 wt CDRH1 codon optimized
gggaggatcttcaggagcttctac

SEQ ID NO: 73 - DNA, 24 bp, Artificial Sequence
  Synthetic sequence HBC34 wt CDRH2 codon optimized
atcaaccaggacggatctgaaaag

SEQ ID NO: 74 - DNA, 36 bp, Artificial Sequence
  Synthetic sequence HBC34 wt CDRH3 codon optimized
gccgcttggtctggcaacagcggcgggatggatgtc

SEQ ID NO: 75 - DNA, 18 bp, Artificial Sequence
  Synthetic sequence HBC34 wt CDRL1 codon optimized
aaactgggcaacaagaac

SEQ ID NO: 76 - DNA, 9 bp, Artificial Sequence
  Synthetic sequence HBC34 wt CDRL2 codon optimized
gaggtcaag

SEQ ID NO: 77 - DNA, 27 bp, Artificial Sequence
  Synthetic sequence HBC34 wt CDRL2 long codon optimized
gtcatctacgaggtcaagtatcggcca

SEQ ID NO: 78 - DNA, 27 bp, Artificial Sequence
  Synthetic sequence HBC34 wt CDRL3 codon optimized
cagacttgggattcaactactgtcgtg

SEQ ID NO: 79 - protein, 5 aa, Artificial Sequence
  Synthetic linker sequence
GGSGG

SEQ ID NO: 80 - protein, 7 aa, Hepatitis B Virus
TGPCRTC

SEQ ID NO: 81 - protein, 7 aa, Hepatitis B Virus
GNCTCIP

SEQ ID NO: 82 - protein, 25 aa, Hepatitis B Virus
  discontinuous  epitope mimic
  VARIANT 2, 21, 24: Cysteine coupled to acetamidomethyl
CCIPIPSSWAFGCSTTSTGPCRTCC

SEQ ID NO: 83 - protein, 28 aa, Hepatitis B Virus
  discontinuous epitope mimic
  VARIANT 4,6, 24, 27: Cys is coupled to acetamidomethyl
CGNCTCIPIPSSWAFCSTTSTGPCRTCC

SEQ ID NO: 84 - protein, 17 aa, Hepatitis B Virus
  looped epitope mimic
  VARIANT 13, 16: cys is coupled to acetamidomethyl
CGGGCSTTSTGPCRTCC

SEQ ID NO: 85 - protein, 11 aa, Hepatitis B virus
STTSTGPCRTC

SEQ ID NO: 86 - protein, 15 aa, Hepatitis B Virus
GNCTCIPIPSSWAFC

SEQ ID NO: 87 - protein, 14 aa, Hepatitis B Virus
GNCTCIPIPSSWAF

SEQ ID NO: 88 - protein, 5 aa, Hepatitis B Virus
  VARIANT (1)...(5): Xaa = Any Amino Acid
PCRXC

SEQ ID NO: 89 - protein, 106 aa, Artificial Sequence
  Synthetic sequence HBC34-V35 VL
SYELTQPPSVSVSPGQTVSIPCSGDKLGNKNVAWFQHKPGQSPVLVIYEVKYRPSGIPERFSGSNSGNTATLTISGTQAMDEAAYFCQTFDSTTVVFGGGTRLTVL

SEQ ID NO: 90 - protein, 106 aa, Artificial Sequence
  Synthetic sequence HBC34-V34 VL
SYELTQPPSVSVSPGQTVSIPCSGDKLGNKNVSWFQHKPGQSPVLVIYEVKYRPSGIPERFSGSNSGNTATLTISGTQAMDEAAYFCQTFDSTTVVFGGGTRLTVL

SEQ ID NO: 91 - protein, 449 aa, Artificial Sequence
  Synthetic sequence HC of HBC34-V35-MLNS-GAALIE and HBC34-V34-MLNS-GAALIE (g1M17, 1)
ELQLVESGGGWVQPGGSQRLSCAASGRIFRSFYMSWVRQAPGKGLEWVATINQDGSEKLYVDSVKGRFTISRDNAKNSLFLQMNNLRVEDTAVYYCAAWSGNSGGMDVWGQGTTVSVSSASTKGPSVFPLAPSSKSTSGGTAALGCLVKDYFPEPVTVSWNSGALTSGVHTFPAVLQSSGLYSLSSVVTVPSSSLGTQTYICNVNHKPSNTKVDKKVEPKSCDKTHTCPPCPAPELLAGPSVFLFPPKPKDTLMISRTPEVTCVVVDVSHEDPEVKFNWYVDGVEVHNAKTKPREEQYNSTYRVVSVLTVLHQDWLNGKEYKCKVSNKALPLPEEKTISKAKGQPREPQVYTLPPSRDELTKNQVSLTCLVKGFYPSDIAVEWESNGQPENNYKTTPPVLDSDGSFFLYSKLTVDKSRWQQGNVFSCSVLHEALHSHYTQKSLSLSPGK

SEQ ID NO: 92 - protein, 449 aa, Artificial Sequence
  Synthetic sequence HC of HBC34-V35-MLNS and HBC34-V34-MLNS (g1M17, 1)
ELQLVESGGGWVQPGGSQRLSCAASGRIFRSFYMSWVRQAPGKGLEWVATINQDGSEKLYVDSVKGRFTISRDNAKNSLFLQMNNLRVEDTAVYYCAAWSGNSGGMDVWGQGTTVSVSSASTKGPSVFPLAPSSKSTSGGTAALGCLVKDYFPEPVTVSWNSGALTSGVHTFPAVLQSSGLYSLSSVVTVPSSSLGTQTYICNVNHKPSNTKVDKKVEPKSCDKTHTCPPCPAPELLGGPSVFLFPPKPKDTLMISRTPEVTCVVVDVSHEDPEVKFNWYVDGVEVHNAKTKPREEQYNSTYRVVSVLTVLHQDWLNGKEYKCKVSNKALPAPIEKTISKAKGQPREPQVYTLPPSRDELTKNQVSLTCLVKGFYPSDIAVEWESNGQPENNYKTTPPVLDSDGSFFLYSKLTVDKSRWQQGNVFSCSVLHEALHSHYTQKSLSLSPGK

SEQ ID NO: 93 - protein, 212 aa, Artificial Sequence
  Synthetic sequence LC of HBC34-V35
SYELTQPPSVSVSPGQTVSIPCSGDKLGNKNVAWFQHKPGQSPVLVIYEVKYRPSGIPERFSGSNSGNTATLTISGTQAMDEAAYFCQTFDSTTVVFGGGTRLTVLGQPKAAPSVTLFPPSSEELQANKATLVCLISDFYPGAVTVAWKADSSPVKAGVETTTPSKQSNNKYAASSYLSLTPEQWKSHRSYSCQVTHEGSTVEKTVAPTECS

SEQ ID NO: 94 - protein, 212 aa, Artificial Sequence
  Synthetic sequence LC of HBC34-V34
SYELTQPPSVSVSPGQTVSIPCSGDKLGNKNVSWFQHKPGQSPVLVIYEVKYRPSGIPERFSGSNSGNTATLTISGTQAMDEAAYFCQTFDSTTVVFGGGTRLTVLGQPKAAPSVTLFPPSSEELQANKATLVCLISDFYPGAVTVAWKADSSPVKAGVETTTPSKQSNNKYAASSYLSLTPEQWKSHRSYSCQVTHEGSTVEKTVAPTECS

SEQ ID NO: 95 - protein, 128 aa, Artificial Sequence
  Synthetic sequence HBC24 VH
EVQLLESGGGLVQPGGSLRLSCAASGSTFTKYAMSWVRQAPGKGLEWVASISGSVPGFGIDTYYADSVKGRFTISRDTSKNTLYLQMNSLRAEDTALYYCAKDVGVIGSYYYYAMDVWGQGTAVTVSS

SEQ ID NO: 96 - protein, 109 aa, Artificial Sequence
  Synthetic sequence HBC24 VL
EIVLTQSPGTLSLSPGERATLSCRASQGLSSSYLAWYQQKPGQAPRLLIYSASTRATGIPDRFSGSGSGTDFTLTISRLEPEDFAVYYCQQYAYSPRWTFGQGTKVEIK

SEQ ID NO: 97 - protein, 8 aa, Artificial Sequence
  Synthetic sequence CDRH1 of HBC24
GSTFTKYA

SEQ ID NO: 98 - protein, 8 aa, Artificial Sequence
  Synthetic sequence CDRH2 of HBC24
ISGSVPGF

SEQ ID NO: 99 - protein, 21 aa, Artificial Sequence
  Synthetic sequence CDRH3 of HBC24
LYYCAKDVGVIGSYYYYAMDV

SEQ ID NO: 100 - protein, 7 aa, Artificial Sequence
  Synthetic sequence CDRL1 of HBC24
QGLSSSY

SEQ ID NO: 101 - protein, 3 aa, Artificial Sequence
  Synthetic sequence CDRL2 of HBC24
SAS

SEQ ID NO: 102 - protein, 10 aa, Artificial Sequence
  Synthetic sequence CDRL3 of HBC24
QQYAYSPRWT

SEQ ID NO: 103 - DNA, 357 bp, Artificial Sequence
  Synthetic sequence VH of  HBC34-V7, HBC34-V35, and HBC34-V34 (codon optimized)
gagctgcagctggtggagtccggcggcggctgggtgcagcctggcggctcccagaggctgagctgtgccgcttctggcaggatcttccggtccttttacatgtcttgggtgcggcaggctccaggcaagggcctggagtgggtggctaccatcaaccaggacggctccgagaagctgtatgtggatagcgtgaagggcagattcacaatctctcgcgacaacgccaagaactccctgtttctgcagatgaacaatctgagggtggaggataccgccgtgtactattgcgccgcttggtctggcaatagcggcggcatggacgtgtggggacagggcaccaccgtgtccgtgtccagc

SEQ ID NO: 104 - DNA, 318 bp, Artificial Sequence
  Synthetic sequence HBC34-V34 VL (codon optimized)
agctacgagctgacacagcccccttccgtgtccgtgtcccctggacagaccgtgtccatcccatgcagcggcgacaagctgggcaacaagaacgtgtcctggtttcagcataagcctggccagtcccccgtgctggtcatctacgaggtgaagtataggcccagcggcatccctgagcggttctctggctccaacagcggcaatacagccaccctgacaatctctggcacacaggctatggacgaggccgcttatttctgccagacctttgattccaccacagtggtgttcggcggcggcaccagactgacagtgctg

SEQ ID NO: 105 - DNA, 318 bp, Artificial Sequence
  Synthetic sequence HBC34-V35 VL (codon optimized)
agctacgagctgacacagcccccttccgtgtccgtgtcccctggacagaccgtgtccatcccatgcagcggcgacaagctgggcaacaagaacgtggcctggtttcagcataagcctggccagtcccccgtgctggtcatctacgaggtgaagtataggcccagcggcatccctgagcggttctctggctccaacagcggcaatacagccaccctgacaatctctggcacacaggctatggacgaggccgcttatttctgccagacctttgattccaccacagtggtgttcggcggcggcaccagactgacagtgctg

SEQ ID NO: 106 - DNA, 360 bp, Artificial Sequence
  Synthetic sequence HBC24 VH (wild type)
gaggtgcagttgttggagtctgggggaggcttggtacagcctggggggtccctgagactctcctgtgcagcctctggatccacttttaccaaatatgccatgagctgggtccgtcaggctccagggaaggggctggagtgggtcgcaagtattagtggaagtgttcctggttttggtattgacacatactacgcagactccgttaagggccggttcaccatctccagagacacttccaagaacaccctgtatctgcaaatgaacagcctgagagccgaggacacggccttatattactgtgcgaaagatgtcggggttatcgggtcatactattactacgctatggacgtctggggtcaa

SEQ ID NO: 107 - DNA, 327 bp, Artificial Sequence
  Synthetic sequence HBC24 VL (wild type)
aaattgtgttgacgcagtctccaggcaccctgtctttgtctccaggggaaagagccaccctctcctgcagggccagtcagggtcttagcagcagttacttagcctggtaccagcagaaacctggccaggctcccaggctcctcatctatagtgcgtccaccagggccactggcatcccagacaggttcagtggcagtgggtctgggacagacttcactctcaccatcagcagactggagcctgaagattttgcagtgtattactgtcaacagtatgcttactcacctcggtggacgttcggccaagggaccaaggtggagatcaaac

SEQ ID NO: 108 - DNA, 384 bp, Artificial Sequence
  Synthetic sequence HBC24 VH (codon optimized)
gaggtgcagctgctggaaagcggcggcggcctggtgcagcccggcggctccctgaggctgtcttgcgccgcctctggcagcaccttcacaaagtatgcaatgtcttgggtgcgccaggcaccaggcaagggcctggagtgggtggcctccatctctggcagcgtgcctggcttcggcatcgacacctactatgccgattccgtgaagggccggtttacaatcagcagagacacctccaagaacacactgtatctgcagatgaattctctgcgggccgaggacaccgccctgtactattgtgccaaggatgtgggcgtgatcggcagctactattactatgcaatggacgtgtggggacagggaacagcagtgacagtgagctcc

SEQ ID NO: 109 - DNA, 327 bp, Artificial Sequence
  Synthetic sequence HBC24 VL (codon optimized)
gagatcgtgctgacccagtctcctggcacactgtccctgtcccctggagagagagccaccctgtcctgcagagcctctcagggcctgagctcctcttacctggcctggtatcagcagaagcctggacaggcccctcggctgctgatctactctgcctccaccagagcaacaggcattcctgaccgcttctccggatctggaagcggcacagacttcaccctgacaatcagccggctggagcctgaggacttcgccgtgtactattgtcagcagtacgcctattccccaaggtggacctttggccagggcacaaaggtggagatcaag

SEQ ID NO: 110 - DNA, 318 bp, Artificial Sequence
  Synthetic sequence HBC34-V7 VL (codon optimized)
agctacgagctgacacagcccccttccgtgtccgtgtcccctggacagaccgtgtccatcccatgcagcggcgacaagctgggcaacaagaacgtgtgctggtttcagcataagcctggccagtcccccgtgctggtcatctacgaggtgaagtataggcccagcggcatccctgagcggttctctggctccaacagcggcaatacagccaccctgacaatctctggcacacaggctatggacgaggccgcttatttctgccagacctttgattccaccacagtggtgttcggcggcggcaccagactgacagtgctg

SEQ ID NO: 111 - protein, 106 aa, Artificial Sequence
  Synthetic sequence HBC34v23-L_C40S
SYELTQPPSVSVSPGQTASITCSGDKLGNKNASWYQQKPGQSPVLVIYEVKYRPSGIPERFSGSNSGNTATLTISGTQAMDEADYYCQTFDSTTVVFGGGTKLTVL

SEQ ID NO: 112 - protein, 106 aa, Artificial Sequence
  Synthetic sequence HBC34v23-L_C40A
SYELTQPPSVSVSPGQTASITCSGDKLGNKNAAWYQQKPGQSPVLVIYEVKYRPSGIPERFSGSNSGNTATLTISGTQAMDEADYYCQTFDSTTVVFGGGTKLTVL

SEQ ID NO: 113 - protein, 106 aa, Artificial Sequence
  Synthetic sequence HBC34v31-L_C40S
SYELTQPPSVSVSPGQTVSIPCSGDKLGNKNVSWFQHKPGQSPVLVIYEVKYRPSGIPERFSGSNSGNTATLTISGTQAMDEAAYFCQTWDSTTVVFGGGTRLTVL

SEQ ID NO: 114 - protein, 106 aa, Artificial Sequence
  Synthetic sequence HBC34v31-L_C40A
SYELTQPPSVSVSPGQTVSIPCSGDKLGNKNVAWFQHKPGQSPVLVIYEVKYRPSGIPERFSGSNSGNTATLTISGTQAMDEAAYFCQTWDSTTVVFGGGTRLTVL

SEQ ID NO: 115 - protein, 106 aa, Artificial Sequence; identical to SEQ ID NO: 90
  Synthetic sequence HBC34v32-L_C40S

SEQ ID NO: 116 - protein, 106 aa, Artificial Sequence; identical to SEQ ID NO: 114
  Synthetic sequence HBC34v32-L_C40A

SEQ ID NO: 117 - protein, 106 aa, Artificial Sequence; identical to SEQ ID NO: 111
  Synthetic sequence HBC34v33-L_C40S

SEQ ID NO: 118 - protein, 106 aa, Artificial Sequence; identical to SEQ ID NO: 112
  Synthetic sequence HBC34v33-L_C40A

SEQ ID NO: 119 - protein, 106 aa, Artificial Sequence; identical to SEQ ID NO: 113
  Synthetic sequence HBC34-L_C40S

SEQ ID NO: 120 - protein, 106 aa, Artificial Sequence; identical to SEQ ID NO: 114
  Synthetic sequence HBC34-L_C40A

SEQ ID NO: 121 - protein, 458 aa, Artificial Sequence
  Synthetic sequence HBC24-MLNS
EVQLLESGGGLVQPGGSLRLSCAASGSTFTKYAMSWVRQAPGKGLEWVASISGSVPGFGIDTYYADSVKGRFTISRDTSKNTLYLQMNSLRAEDTALYYCAKDVGVIGSYYYYAMDVWGQGTAVTVSSASTKGPSVFPLAPSSKSTSGGTAALGCLVKDYFPEPVTVSWNSGALTSGVHTFPAVLQSSGLYSLSSVVTVPSSSLGTQTYICNVNHKPSNTKVDKKVEPKSCDKTHTCPPCPAPELLGGPSVFLFPPKPKDTLMISRTPEVTCVVVDVSHEDPEVKFNWYVDGVEVHNAKTKPREEQYNSTYRVVSVLTVLHQDWLNGKEYKCKVSNKALPAPIEKTISKAKGQPREPQVYTLPPSRDELTKNQVSLTCLVKGFYPSDIAVEWESNGQPENNYKTTPPVLDSDGSFFLYSKLTVDKSRWQQGNVFSCSVLHEALHSHYTQKSLSLSPGK

SEQ ID NO: 122 - protein, 458 aa, Artificial Sequence
  Synthetic sequence HBC24-MLNS-GAALIE
EVQLLESGGGLVQPGGSLRLSCAASGSTFTKYAMSWVRQAPGKGLEWVASISGSVPGFGIDTYYADSVKGRFTISRDTSKNTLYLQMNSLRAEDTALYYCAKDVGVIGSYYYYAMDVWGQGTAVTVSSASTKGPSVFPLAPSSKSTSGGTAALGCLVKDYFPEPVTVSWNSGALTSGVHTFPAVLQSSGLYSLSSVVTVPSSSLGTQTYICNVNHKPSNTKVDKKVEPKSCDKTHTCPPCPAPELLAGPSVFLFPPKPKDTLMISRTPEVTCVVVDVSHEDPEVKFNWYVDGVEVHNAKTKPREEQYNSTYRVVSVLTVLHQDWLNGKEYKCKVSNKALPLPEEKTISKAKGQPREPQVYTLPPSRDELTKNQVSLTCLVKGFYPSDIAVEWESNGQPENNYKTTPPVLDSDGSFFLYSKLTVDKSRWQQGNVFSCSVLHEALHSHYTQKSLSLSPGK

SEQ ID NO: 123 - protein, 449 aa, Artificial Sequence
  Synthetic sequence HBC34-V7-mu (IgG2a) HC
ELQLVESGGGWVQPGGSQRLSCAASGRIFRSFYMSWVRQAPGKGLEWVATINQDGSEKLYVDSVKGRFTISRDNAKNSLFLQMNNLRVEDTAVYYCAAWSGNSGGMDVWGQGTTVSVSSAKTTAPSVYPLAPVCGDTTGSSVTLGCLVKGYFPEPVTLTWNSGSLSSGVHTFPAVLQSDLYTLSSSVTVTSSTWPSQSITCNVAHPASSTKVDKKIEPRGPTIKPCPPCKCPAPNLLGGPSVFIFPPKIKDVLMISLSPIVTCVVVDVSEDDPDVQISWFVNNVEVHTAQTQTHREDYNSTLRVVSALPIQHQDWMSGKEFKCKVNNKDLPAPIERTISKPKGSVRAPQVYVLPPPEEEMTKKQVTLTCMVTDFMPEDIYVEWTNNGKTELNYKNTEPVLDSDGSYFMYSKLRVEKKNWVERNSYSCSVVHEGLHNHHTTKSFSRTPGK

SEQ ID NO: 124 - protein, 212 aa, Artificial Sequence
  Synthetic sequence HBC34-V7-mu (IgG2a) LC
SYELTQPPSVSVSPGQTVSIPCSGDKLGNKNVCWFQHKPGQSPVLVIYEVKYRPSGIPERFSGSNSGNTATLTISGTQAMDEAAYFCQTFDSTTVVFGGGTRLTVLGQPKSSPSVTLFPPSSEELETNKATLVCTITDFYPGVVTVDWKVDGTPVTQGMETTQPSKQSNNKYMASSYLTLTARAWERHSSYSCQVTHEGHTVEKSLSRADCS

SEQ ID NO: 125 - protein, 449 aa, Artificial Sequence; identical to SEQ ID NO: 123
  Synthetic sequence HBC34-V35-mu (IgG2a) HC

SEQ ID NO: 126 - protein, 212 aa, Artificial Sequence
  Synthetic sequence HBC34-V35-mu (IgG2a) LC
SYELTQPPSVSVSPGQTVSIPCSGDKLGNKNVAWFQHKPGQSPVLVIYEVKYRPSGIPERFSGSNSGNTATLTISGTQAMDEAAYFCQTFDSTTVVFGGGTRLTVLGQPKSSPSVTLFPPSSEELETNKATLVCTITDFYPGVVTVDWKVDGTPVTQGMETTQPSKQSNNKYMASSYLTLTARAWERHSSYSCQVTHEGHTVEKSLSRADCS

SEQ ID NO: 127 - protein, 458 aa, Artificial Sequence
  Synthetic sequence HBC24-mu (IgG2a) HC
EVQLLESGGGLVQPGGSLRLSCAASGSTFTKYAMSWVRQAPGKGLEWVASISGSVPGFGIDTYYADSVKGRFTISRDTSKNTLYLQMNSLRAEDTALYYCAKDVGVIGSYYYYAMDVWGQGTAVTVSSAKTTAPSVYPLAPVCGDTTGSSVTLGCLVKGYFPEPVTLTWNSGSLSSGVHTFPAVLQSDLYTLSSSVTVTSSTWPSQSITCNVAHPASSTKVDKKIEPRGPTIKPCPPCKCPAPNLLGGPSVFIFPPKIKDVLMISLSPIVTCVVVDVSEDDPDVQISWFVNNVEVHTAQTQTHREDYNSTLRVVSALPIQHQDWMSGKEFKCKVNNKDLPAPIERTISKPKGSVRAPQVYVLPPPEEEMTKKQVTLTCMVTDFMPEDIYVEWTNNGKTELNYKNTEPVLDSDGSYFMYSKLRVEKKNWVERNSYSCSVVHEGLHNHHTTKSFSRTPGK

SEQ ID NO: 128 - protein, 215 aa, Artificial Sequence
  Synthetic sequence HBC24-mu (IgG2a) LC
EIVLTQSPGTLSLSPGERATLSCRASQGLSSSYLAWYQQKPGQAPRLLIYSASTRATGIPDRFSGSGSGTDFTLTISRLEPEDFAVYYCQQYAYSPRWTFGQGTKVEIKADAAPTVSIFPPSSEQLTSGGASVVCFLNNFYPKDINVKWKIDGSERQNGVLNSWTDQDSKDSTYSMSSTLTLTKDEYERHNSYTCEATHKTSTSPIVKSFNRNEC

SEQ ID NO: 129 - protein, 449 aa, Artificial Sequence
  Synthetic sequence HBC34-V7, HBC34-V34, HBC34-V35 HC (wild-type)
ELQLVESGGGWVQPGGSQRLSCAASGRIFRSFYMSWVRQAPGKGLEWVATINQDGSEKLYVDSVKGRFTISRDNAKNSLFLQMNNLRVEDTAVYYCAAWSGNSGGMDVWGQGTTVSVSSASTKGPSVFPLAPSSKSTSGGTAALGCLVKDYFPEPVTVSWNSGALTSGVHTFPAVLQSSGLYSLSSVVTVPSSSLGTQTYICNVNHKPSNTKVDKKVEPKSCDKTHTCPPCPAPELLGGPSVFLFPPKPKDTLMISRTPEVTCVVVDVSHEDPEVKFNWYVDGVEVHNAKTKPREEQYNSTYRVVSVLTVLHQDWLNGKEYKCKVSNKALPAPIEKTISKAKGQPREPQVYTLPPSRDELTKNQVSLTCLVKGFYPSDIAVEWESNGQPENNYKTTPPVLDSDGSFFLYSKLTVDKSRWQQGNVFSCSVMHEALHNHYTQKSLSLSPGK

SEQ ID NO: 130 - DNA, 990 bp, Artificial Sequence
  Synthetic sequence HBC34-V7, HBC34-V34, HBC34-V35 CH1-hinge-CH2-CH3 (codon-optimized)
gcctccacaaagggcccaagcgtgtttccactggctccctcttccaagtctacctccggcggcacagccgctctgggatgtctggtgaaggattacttcccagagcccgtgaccgtgtcttggaactccggcgccctgaccagcggagtgcatacatttccagctgtgctgcagagctctggcctgtactctctgtccagcgtggtgaccgtgccctcttccagcctgggcacccagacatatatctgcaacgtgaatcacaagccaagcaatacaaaggtggacaagaaggtggagcccaagtcttgtgataagacccatacatgccctccatgtccagctccagagctgctgggcggcccaagcgtgttcctgtttccacccaagcctaaggataccctgatgatctccagaacccccgaggtgacatgcgtggtggtggacgtgagccacgaggatcctgaggtgaagttcaactggtacgtggacggcgtggaggtgcataatgctaagaccaagcccagggaggagcagtacaactctacctatcgggtggtgtccgtgctgacagtgctgcaccaggattggctgaacggcaaggagtataagtgcaaggtgtctaataaggccctgcccgctcctatcgagaagaccatctccaaggccaagggccagcctagagagccacaggtgtacacactgcctccatctcgcgatgagctgaccaagaaccaggtgtccctgacatgtctggtgaagggcttctatccttccgacatcgctgtggagtgggagagcaatggccagccagagaacaattacaagaccacaccccctgtgctggacagcgatggctctttctttctgtatagcaagctgaccgtggacaagtctcgctggcagcagggcaacgtgtttagctgttctgtgatgcatgaggccctgcacaatcattatacacagaagtccctgagcctgtctcctggcaag

SEQ ID NO: 131 - DNA, 1417 bp, Artificial Sequence
  Synthetic sequence HBC34-V7, HBC34-V34, HBC34-V35 VH-CH1-hinge-CH2-CH3 (codon-optimized)
gagctgcagctggtggagtccggcggcggctgggtgcagcctggcggctcccagaggctgagctgtgccgcttctggcaggatcttccggtccttttacatgtcttgggtgcggcaggctccaggcaagggcctggagtgggtggctaccatcaaccaggacggctccgagaagctgtatgtggatagcgtgaagggcagattcacaatctctcgcgacaacgccaagaactccctgtttctgcagatgaacaatctgagggtggaggataccgccgtgtactattgcgccgcttggtctggcaatagcggcggcatggacgtgtggggacagggcaccaccgtgtccgtgtccagcgcctccacaaagggcccaagcgtgtttccactggctccctcttccaagtctacctccggcggcacagccgctctgggatgtctggtgaaggattacttcccagagcccgtgaccgtgtcttggaactccggcgccctgaccagcggagtgcatacatttccagctgtgctgcagagctctggcctgtactctctgtccagcgtggtgaccgtgccctcttccagcctgggcacccagacatatatctgcaacgtgaatcacaagccaagcaatacaaaggtggacaagaaggtggagcccaagtcttgtgataagacccatacatgccctccatgtccagctccagagctgctgggcggcccaagcgtgttcctgtttccacccaagcctaaggataccctgatgatctccagaacccccgaggtgacatgcgtggtggtggacgtgagccacgaggatcctgaggtgaagttcaactggtacgtggacggcgtggaggtgcataatgctaagaccaagcccagggaggagcagtacaactctacctatcgggtggtgtccgtgctgacagtgctgcaccaggattggctgaacggcaaggagtataagtgcaaggtgtctaataaggccctgcccgctcctatcgagaagaccatctccaaggccaagggccagcctagagagccacaggtgtacacactgcctccatctcgcgatgagctgaccaagaaccaggtgtccctgacatgtctggtgaagggcttctatccttccgacatcgctgtggagtgggagagcaatggccagccagagaacaattacaagaccacaccccctgtgctggacagcgatggctctttctttctgtatagcaagctgaccgtggacaagtctcgctggcagcagggcaacgtgtttagctgttctgtgatgcatgaggccctgcacaatcattatacacagaagtccctgagcctgtctcctggcaagtgatgaggtaccgtgcgacggccggcaagcccccgctccccgggctctcgcggtcgtacgaggaaagctt

SEQ ID NO: 132 - DNA, 318 bp, Artificial Sequence
  Synthetic sequence HBC34-V7 CL (codon-optimized)
ggacagccaaaggctgctccatctgtgaccctgtttccaccctcttccgaggagctgcaggccaacaaggccaccctggtgtgcctgatctctgacttctaccctggagctgtgacagtggcttggaaggctgatagctctcccgtgaaggctggcgtggagacaacaacccctagcaagcagtctaacaataagtacgccgcttccagctatctgtctctgacaccagagcagtggaagtcccaccgctcttattcctgccaggtgacccatgagggcagcaccgtggagaagacagtggcccccaccgagtgttct

SEQ ID NO: 133 - DNA, 636 bp, Artificial Sequence
  Synthetic sequence HBC34-V7 LC (VL-CL) (codon-optimized)
agctacgagctgacacagcccccttccgtgtccgtgtcccctggacagaccgtgtccatcccatgcagcggcgacaagctgggcaacaagaacgtgtgctggtttcagcataagcctggccagtcccccgtgctggtcatctacgaggtgaagtataggcccagcggcatccctgagcggttctctggctccaacagcggcaatacagccaccctgacaatctctggcacacaggctatggacgaggccgcttatttctgccagacctttgattccaccacagtggtgttcggcggcggcaccagactgacagtgctgggacagccaaaggctgctccatctgtgaccctgtttccaccctcttccgaggagctgcaggccaacaaggccaccctggtgtgcctgatctctgacttctaccctggagctgtgacagtggcttggaaggctgatagctctcccgtgaaggctggcgtggagacaacaacccctagcaagcagtctaacaataagtacgccgcttccagctatctgtctctgacaccagagcagtggaagtcccaccgctcttattcctgccaggtgacccatgagggcagcaccgtggagaagacagtggcccccaccgagtgttct

SEQ ID NO: 134 - DNA, 318 bp, Artificial Sequence; identical to SEQ ID NO: 132
  Synthetic sequence HBC34-V34,  HBC34-V35 CL (codon-optimized)

SEQ ID NO: 135 - DNA, 636 bp, Artificial Sequence
  Synthetic sequence HBC34-V34 LC (VL-CL) (codon-optimized)
agctacgagctgacacagcccccttccgtgtccgtgtcccctggacagaccgtgtccatcccatgcagcggcgacaagctgggcaacaagaacgtgtcctggtttcagcataagcctggccagtcccccgtgctggtcatctacgaggtgaagtataggcccagcggcatccctgagcggttctctggctccaacagcggcaatacagccaccctgacaatctctggcacacaggctatggacgaggccgcttatttctgccagacctttgattccaccacagtggtgttcggcggcggcaccagactgacagtgctgggacagccaaaggctgctccatctgtgaccctgtttccaccctcttccgaggagctgcaggccaacaaggccaccctggtgtgcctgatctctgacttctaccctggagctgtgacagtggcttggaaggctgatagctctcccgtgaaggctggcgtggagacaacaacccctagcaagcagtctaacaataagtacgccgcttccagctatctgtctctgacaccagagcagtggaagtcccaccgctcttattcctgccaggtgacccatgagggcagcaccgtggagaagacagtggcccccaccgagtgttct

SEQ ID NO: 136 - DNA, 636 bp, Artificial Sequence
  Synthetic sequence HBC34-V35 LC (VL-CL) (codon-optimized)
agctacgagctgacacagcccccttccgtgtccgtgtcccctggacagaccgtgtccatcccatgcagcggcgacaagctgggcaacaagaacgtggcctggtttcagcataagcctggccagtcccccgtgctggtcatctacgaggtgaagtataggcccagcggcatccctgagcggttctctggctccaacagcggcaatacagccaccctgacaatctctggcacacaggctatggacgaggccgcttatttctgccagacctttgattccaccacagtggtgttcggcggcggcaccagactgacagtgctgggacagccaaaggctgctccatctgtgaccctgtttccaccctcttccgaggagctgcaggccaacaaggccaccctggtgtgcctgatctctgacttctaccctggagctgtgacagtggcttggaaggctgatagctctcccgtgaaggctggcgtggagacaacaacccctagcaagcagtctaacaataagtacgccgcttccagctatctgtctctgacaccagagcagtggaagtcccaccgctcttattcctgccaggtgacccatgagggcagcaccgtggagaagacagtggcccccaccgagtgttct

SEQ ID NO: 137 - protein, 217 aa, Homo sapiens IgG1
  WT hIgG1 Fc
APELLGGPSVFLFPPKPKDTLMISRTPEVTCVVVDVSHEDPEVKFNWYVDGVEVHNAKTKPREEQYNSTYRVVSVLTVLHQDWLNGKEYKCKVSNKALPAPIEKTISKAKGQPREPQVYTLPPSRDELTKNQVSLTCLVKGFYPSDIAVEWESNGQPENNYKTTPPVLDSDGSFFLYSKLTVDKSRWQQGNVFSCSVMHEALHNHYTQKSLSLSPGK

SEQ ID NO: 138 - protein, 449 aa, Artificial Sequence
  Synthetic sequence HBC34, HBC34v7, HBC34v23, HBC34v34, HBC34v35, HBC34_C40S, HBC34_C40A, HBC34v23_C40S, HBC34v23_C40A HC with GAALIE mutation in hIgG1 Fc
ELQLVESGGGWVQPGGSQRLSCAASGRIFRSFYMSWVRQAPGKGLEWVATINQDGSEKLYVDSVKGRFTISRDNAKNSLFLQMNNLRVEDTAVYYCAAWSGNSGGMDVWGQGTTVSVSSASTKGPSVFPLAPSSKSTSGGTAALGCLVKDYFPEPVTVSWNSGALTSGVHTFPAVLQSSGLYSLSSVVTVPSSSLGTQTYICNVNHKPSNTKVDKKVEPKSCDKTHTCPPCPAPELLAGPSVFLFPPKPKDTLMISRTPEVTCVVVDVSHEDPEVKFNWYVDGVEVHNAKTKPREEQYNSTYRVVSVLTVLHQDWLNGKEYKCKVSNKALPLPEEKTISKAKGQPREPQVYTLPPSRDELTKNQVSLTCLVKGFYPSDIAVEWESNGQPENNYKTTPPVLDSDGSFFLYSKLTVDKSRWQQGNVFSCSVMHEALHNHYTQKSLSLSPGK

SEQ ID NO: 139 - protein, 19 aa, Artificial Sequence
  Chimeric hinge sequence
ESKYGPPCPPCPAPPVAGP